European Patent Application EP 4 458 961 A1, published November 6, 2024. Title: ISOLATED POLYPEPTIDE AND USE THEREOF. Applicant: GLYCO-THERAPY BIOTECHNOLOGY CO., LTD. The sequence listing filed with the application follows.

SEQUENCE LISTING (30 sequences)

SEQ ID NO: 1 - protein, 364 aa, Artificial Sequence
  1-364 of the Helicobacter pylori alfa(1,3)-fucosyltransferase (GenBank No. AAD07710.1)
MFQPLLDAFIESASIEKMVSKSPPPPLKIAVANWWGDEEIKEFKKSVLYFILSQRYAITLHQNPNESSDLVFSNPLGAARKILSYQNTKRVFYTGENESPNFNLFDYAIGFDELDFNDRYLRMPLYYAHLHYEAELVNDTTAPYKLKDNSLYALKKPSHHFKENHPNLCAVVNDESDLLKRGFASFVASNANAPMRNAFYDALNSIEPVTGGGSVRNTLGYKVGNKSEFLSQYKFNLCFENSQGYGYVTEKILDAYFSHTIPIYWGSPSVAKDFNPKSFVNVHDFNNFDEAIDYIKYLHTHPNAYLDMLYENPLNTLDGKAYFYQDLSFKKILDFFKTILENDTIYHNNPFIFYRDLHEPLISI

SEQ ID NO: 2 - protein, 7 aa, Artificial Sequence
  Heptapeptide repeat sequence (HR) of Helicobacter pylori alfa-1,3 fucosyltransferase (GenBank No. AAD07710.1)
DDLRVNY

SEQ ID NO: 3 - protein, 371 aa, Artificial Sequence
  Catalytically active domain of Helicobacter pylori alfa-1,3 fucosyltransferase(GenBank No.AAD07710.1) with 1 heptapeptide repeat
MFQPLLDAFIESASIEKMVSKSPPPPLKIAVANWWGDEEIKEFKKSVLYFILSQRYAITLHQNPNESSDLVFSNPLGAARKILSYQNTKRVFYTGENESPNFNLFDYAIGFDELDFNDRYLRMPLYYAHLHYEAELVNDTTAPYKLKDNSLYALKKPSHHFKENHPNLCAVVNDESDLLKRGFASFVASNANAPMRNAFYDALNSIEPVTGGGSVRNTLGYKVGNKSEFLSQYKFNLCFENSQGYGYVTEKILDAYFSHTIPIYWGSPSVAKDFNPKSFVNVHDFNNFDEAIDYIKYLHTHPNAYLDMLYENPLNTLDGKAYFYQDLSFKKILDFFKTILENDTIYHNNPFIFYRDLHEPLISIDDLRVNY

SEQ ID NO: 4 - protein, 378 aa, Artificial Sequence
  Catalytically active domain of Helicobacter pylori alfa-1,3 fucosyltransferase(GenBank No.AAD07710.1) with 2 heptapeptide repeats
MFQPLLDAFIESASIEKMVSKSPPPPLKIAVANWWGDEEIKEFKKSVLYFILSQRYAITLHQNPNESSDLVFSNPLGAARKILSYQNTKRVFYTGENESPNFNLFDYAIGFDELDFNDRYLRMPLYYAHLHYEAELVNDTTAPYKLKDNSLYALKKPSHHFKENHPNLCAVVNDESDLLKRGFASFVASNANAPMRNAFYDALNSIEPVTGGGSVRNTLGYKVGNKSEFLSQYKFNLCFENSQGYGYVTEKILDAYFSHTIPIYWGSPSVAKDFNPKSFVNVHDFNNFDEAIDYIKYLHTHPNAYLDMLYENPLNTLDGKAYFYQDLSFKKILDFFKTILENDTIYHNNPFIFYRDLHEPLISIDDLRVNYDDLRVNY

SEQ ID NO: 5 - protein, 385 aa, Artificial Sequence
  Catalytically active domain of Helicobacter pylori alfa-1,3 fucosyltransferase(GenBank No.AAD07710.1) with 3 heptapeptide repeats
MFQPLLDAFIESASIEKMVSKSPPPPLKIAVANWWGDEEIKEFKKSVLYFILSQRYAITLHQNPNESSDLVFSNPLGAARKILSYQNTKRVFYTGENESPNFNLFDYAIGFDELDFNDRYLRMPLYYAHLHYEAELVNDTTAPYKLKDNSLYALKKPSHHFKENHPNLCAVVNDESDLLKRGFASFVASNANAPMRNAFYDALNSIEPVTGGGSVRNTLGYKVGNKSEFLSQYKFNLCFENSQGYGYVTEKILDAYFSHTIPIYWGSPSVAKDFNPKSFVNVHDFNNFDEAIDYIKYLHTHPNAYLDMLYENPLNTLDGKAYFYQDLSFKKILDFFKTILENDTIYHNNPFIFYRDLHEPLISIDDLRVNYDDLRVNYDDLRVNY

SEQ ID NO: 6 - protein, 392 aa, Artificial Sequence
  Catalytically active domain of Helicobacter pylori alfa-1,3 fucosyltransferase(GenBank No.AAD07710.1) with 4 heptapeptide repeats
MFQPLLDAFIESASIEKMVSKSPPPPLKIAVANWWGDEEIKEFKKSVLYFILSQRYAITLHQNPNESSDLVFSNPLGAARKILSYQNTKRVFYTGENESPNFNLFDYAIGFDELDFNDRYLRMPLYYAHLHYEAELVNDTTAPYKLKDNSLYALKKPSHHFKENHPNLCAVVNDESDLLKRGFASFVASNANAPMRNAFYDALNSIEPVTGGGSVRNTLGYKVGNKSEFLSQYKFNLCFENSQGYGYVTEKILDAYFSHTIPIYWGSPSVAKDFNPKSFVNVHDFNNFDEAIDYIKYLHTHPNAYLDMLYENPLNTLDGKAYFYQDLSFKKILDFFKTILENDTIYHNNPFIFYRDLHEPLISIDDLRVNYDDLRVNYDDLRVNYDDLRVNY

SEQ ID NO: 7 - protein, 372 aa, Artificial Sequence
  Catalytically active domain of Helicobacter pylori alfa-1,3 fucosyltransferase(GenBank No.AAD07710.1) with a  C-terminal His tag
MFQPLLDAFIESASIEKMVSKSPPPPLKIAVANWWGDEEIKEFKKSVLYFILSQRYAITLHQNPNESSDLVFSNPLGAARKILSYQNTKRVFYTGENESPNFNLFDYAIGFDELDFNDRYLRMPLYYAHLHYEAELVNDTTAPYKLKDNSLYALKKPSHHFKENHPNLCAVVNDESDLLKRGFASFVASNANAPMRNAFYDALNSIEPVTGGGSVRNTLGYKVGNKSEFLSQYKFNLCFENSQGYGYVTEKILDAYFSHTIPIYWGSPSVAKDFNPKSFVNVHDFNNFDEAIDYIKYLHTHPNAYLDMLYENPLNTLDGKAYFYQDLSFKKILDFFKTILENDTIYHNNPFIFYRDLHEPLISILEHHHHHH

SEQ ID NO: 8 - protein, 379 aa, Artificial Sequence
  Catalytically active domain of Helicobacter pylori alfa-1,3 fucosyltransferase(GenBank No.AAD07710.1) with 1 heptapeptide repeat and a C-terminal His tag
MFQPLLDAFIESASIEKMVSKSPPPPLKIAVANWWGDEEIKEFKKSVLYFILSQRYAITLHQNPNESSDLVFSNPLGAARKILSYQNTKRVFYTGENESPNFNLFDYAIGFDELDFNDRYLRMPLYYAHLHYEAELVNDTTAPYKLKDNSLYALKKPSHHFKENHPNLCAVVNDESDLLKRGFASFVASNANAPMRNAFYDALNSIEPVTGGGSVRNTLGYKVGNKSEFLSQYKFNLCFENSQGYGYVTEKILDAYFSHTIPIYWGSPSVAKDFNPKSFVNVHDFNNFDEAIDYIKYLHTHPNAYLDMLYENPLNTLDGKAYFYQDLSFKKILDFFKTILENDTIYHNNPFIFYRDLHEPLISIDDLRVNYLEHHHHHH

SEQ ID NO: 9 - protein, 386 aa, Artificial Sequence
  Catalytically active domain of Helicobacter pylori alfa-1,3 fucosyltransferase(GenBank No.AAD07710.1) with 2 heptapeptide repeats and a  C-terminal His tag
MFQPLLDAFIESASIEKMVSKSPPPPLKIAVANWWGDEEIKEFKKSVLYFILSQRYAITLHQNPNESSDLVFSNPLGAARKILSYQNTKRVFYTGENESPNFNLFDYAIGFDELDFNDRYLRMPLYYAHLHYEAELVNDTTAPYKLKDNSLYALKKPSHHFKENHPNLCAVVNDESDLLKRGFASFVASNANAPMRNAFYDALNSIEPVTGGGSVRNTLGYKVGNKSEFLSQYKFNLCFENSQGYGYVTEKILDAYFSHTIPIYWGSPSVAKDFNPKSFVNVHDFNNFDEAIDYIKYLHTHPNAYLDMLYENPLNTLDGKAYFYQDLSFKKILDFFKTILENDTIYHNNPFIFYRDLHEPLISIDDLRVNYDDLRVNYLEHHHHHH

SEQ ID NO: 10 - protein, 393 aa, Artificial Sequence
  Catalytically active domain of Helicobacter pylori alfa-1,3 fucosyltransferase(GenBank No.AAD07710.1) with 3 heptapeptide repeats and a C-terminal His tag
MFQPLLDAFIESASIEKMVSKSPPPPLKIAVANWWGDEEIKEFKKSVLYFILSQRYAITLHQNPNESSDLVFSNPLGAARKILSYQNTKRVFYTGENESPNFNLFDYAIGFDELDFNDRYLRMPLYYAHLHYEAELVNDTTAPYKLKDNSLYALKKPSHHFKENHPNLCAVVNDESDLLKRGFASFVASNANAPMRNAFYDALNSIEPVTGGGSVRNTLGYKVGNKSEFLSQYKFNLCFENSQGYGYVTEKILDAYFSHTIPIYWGSPSVAKDFNPKSFVNVHDFNNFDEAIDYIKYLHTHPNAYLDMLYENPLNTLDGKAYFYQDLSFKKILDFFKTILENDTIYHNNPFIFYRDLHEPLISIDDLRVNYDDLRVNYDDLRVNYLEHHHHHH

SEQ ID NO: 11 - protein, 400 aa, Artificial Sequence
  Catalytically active domain of Helicobacter pylori alfa-1,3 fucosyltransferase(GenBank No.AAD07710.1) with 4 heptapeptide repeats and a C-terminal His tag
MFQPLLDAFIESASIEKMVSKSPPPPLKIAVANWWGDEEIKEFKKSVLYFILSQRYAITLHQNPNESSDLVFSNPLGAARKILSYQNTKRVFYTGENESPNFNLFDYAIGFDELDFNDRYLRMPLYYAHLHYEAELVNDTTAPYKLKDNSLYALKKPSHHFKENHPNLCAVVNDESDLLKRGFASFVASNANAPMRNAFYDALNSIEPVTGGGSVRNTLGYKVGNKSEFLSQYKFNLCFENSQGYGYVTEKILDAYFSHTIPIYWGSPSVAKDFNPKSFVNVHDFNNFDEAIDYIKYLHTHPNAYLDMLYENPLNTLDGKAYFYQDLSFKKILDFFKTILENDTIYHNNPFIFYRDLHEPLISIDDLRVNYDDLRVNYDDLRVNYDDLRVNYLEHHHHHH

SEQ ID NO: 12 - protein, 414 aa, Artificial Sequence
  Catalytically active domain of Helicobacter pylori alfa-1,3 fucosyltransferase(GenBank No.AAD07710.1) with 6 heptapeptide repeats and a C-terminal His tag
MFQPLLDAFIESASIEKMVSKSPPPPLKIAVANWWGDEEIKEFKKSVLYFILSQRYAITLHQNPNESSDLVFSNPLGAARKILSYQNTKRVFYTGENESPNFNLFDYAIGFDELDFNDRYLRMPLYYAHLHYEAELVNDTTAPYKLKDNSLYALKKPSHHFKENHPNLCAVVNDESDLLKRGFASFVASNANAPMRNAFYDALNSIEPVTGGGSVRNTLGYKVGNKSEFLSQYKFNLCFENSQGYGYVTEKILDAYFSHTIPIYWGSPSVAKDFNPKSFVNVHDFNNFDEAIDYIKYLHTHPNAYLDMLYENPLNTLDGKAYFYQDLSFKKILDFFKTILENDTIYHNNPFIFYRDLHEPLISIDDLRVNYDDLRVNYDDLRVNYDDLRVNYDDLRVNYDDLRVNYLEHHHHHH

SEQ ID NO: 13 - protein, 400 aa, Artificial Sequence
  Catalytically active domain with S46F/A128N/H129E/Y132I mutations, 4 heptapeptide repeats and a C-terminal His tag
MFQPLLDAFIESASIEKMVSKSPPPPLKIAVANWWGDEEIKEFKKFVLYFILSQRYAITLHQNPNESSDLVFSNPLGAARKILSYQNTKRVFYTGENESPNFNLFDYAIGFDELDFNDRYLRMPLYYNELHIEAELVNDTTAPYKLKDNSLYALKKPSHHFKENHPNLCAVVNDESDLLKRGFASFVASNANAPMRNAFYDALNSIEPVTGGGSVRNTLGYKVGNKSEFLSQYKFNLCFENSQGYGYVTEKILDAYFSHTIPIYWGSPSVAKDFNPKSFVNVHDFNNFDEAIDYIKYLHTHPNAYLDMLYENPLNTLDGKAYFYQDLSFKKILDFFKTILENDTIYHNNPFIFYRDLHEPLISIDDLRVNYDDLRVNYDDLRVNYDDLRVNYLEHHHHHH

SEQ ID NO: 14 - protein, 400 aa, Artificial Sequence
  Catalytically active domain with S46F/A128N/H129E/Y132I/Y200N/E341D/V369A mutations, 4 heptapeptide repeats and a C-terminal His tag
MFQPLLDAFIESASIEKMVSKSPPPPLKIAVANWWGDEEIKEFKKFVLYFILSQRYAITLHQNPNESSDLVFSNPLGAARKILSYQNTKRVFYTGENESPNFNLFDYAIGFDELDFNDRYLRMPLYYNELHIEAELVNDTTAPYKLKDNSLYALKKPSHHFKENHPNLCAVVNDESDLLKRGFASFVASNANAPMRNAFNDALNSIEPVTGGGSVRNTLGYKVGNKSEFLSQYKFNLCFENSQGYGYVTEKILDAYFSHTIPIYWGSPSVAKDFNPKSFVNVHDFNNFDEAIDYIKYLHTHPNAYLDMLYENPLNTLDGKAYFYQDLSFKKILDFFKTILDNDTIYHNNPFIFYRDLHEPLISIDDLRANYDDLRVNYDDLRVNYDDLRVNYLEHHHHHH

SEQ ID NO: 15 - protein, 321 aa, Artificial Sequence
  40-359 of human fucosyltrasferase 6 with a G at N-terminus
GDPTVYPNGSRFPDSTGTPAHSIPLILLWTWPFNKPIALPRCSEMVPGTADCNITADRKVYPQADAVIVHHREVMYNPSAQLPRSSRRQGQRWIWFSMESPSHCWQLKAMDGYFNLTMSYRSDSDIFTPYGWLEPWSGQPAHPPLNLSAKTELVAWAVSNWGPNSARVRYYQSLQAHLKVDVYGRSHKPLPQGTMMETLSRYKFYLAFKNSLHPDYITEKLWRNALEAWAVPVVLGPSRSNYERFLPPDAFIHVDDFQSPKDLARYLQELDKDHARYLSYFRWRETLRPRSFSWALAFCKACWKLQEESRYQTRGIAAWFT

SEQ ID NO: 16 - protein, 287 aa, Artificial Sequence
  130-402 of catalytic domain of bovine alfa-1,4-galactosyltransferase I with Y289L/C342T mutations and a N-terminal tag
MASMTGGQQMGRGSSLTACPEESPLLVGPMLIEFNIPVDLKLVEQQNPKVKLGGRYTPMDCISPHKVAIIIPFRNRQEHLKYWLYYLHPILQRQQLDYGIYVINQAGESMFNRAKLLNVGFKEALKDYDYNCFVFSDVDLIPMNDHNTYRCFSQPRHISVAMDKFGFSLPYVQLFGGVSALSKQQFLSINGFPNNYWGWGGEDDDIYNRLAFRGMSVSRPNAVIGKTRMIRHSRDKKNEPNPQRFDRIAHTKETMLSDGLNSLTYMVLEVQRYPLYTKITVDIGTPS

SEQ ID NO: 17 - protein, 1006 aa, Artificial Sequence
  37-995 of Streptococcus pyogenes Endoglycosidase S  with a N-terminal tag
MHHHHHHSSGLVPRGSGMKETAAAKFERQHMDSPDLGTGGGSGIEGREEKTVQVQKGLPSIDSLHYLSENSKKEFKEELSKAGQESQKVKEILAKAQQADKQAQELAKMKIPEKIPMKPLHGPLYGGYFRTWHDKTSDPTEKDKVNSMGELPKEVDLAFIFHDWTKDYSLFWKELATKHVPKLNKQGTRVIRTIPWRFLAGGDNSGIAEDTSKYPNTPEGNKALAKAIVDEYVYKYNLDGLDVDVEHDSIPKVDKKEDTAGVERSIQVFEEIGKLIGPKGVDKSRLFIMDSTYMADKNPLIERGAPYINLLLVQVYGSQGEKGGWEPVSNRPEKTMEERWQGYSKYIRPEQYMIGFSFYEENAQEGNLWYDINSRKDEDKANGINTDITGTRAERYARWQPKTGGVKGGIFSYAIDRDGVAHQPKKYAKQKEFKDATDNIFHSDYSVSKALKTVMLKDKSYDLIDEKDFPDKALREAVMAQVGTRKGDLERFNGTLRLDNPAIQSLEGLNKFKKLAQLDLIGLSRITKLDRSVLPANMKPGKDTLETVLETYKKDNKEEPATIPPVSLKVSGLTGLKELDLSGFDRETLAGLDAATLTSLEKVDISGNKLDLAPGTENRQIFDTMLSTISNHVGSNEQTVKFDKQKPTGHYPDTYGKTSLRLPVANEKVDLQSQLLFGTVTNQGTLINSEADYKAYQNHKIAGRSFVDSNYHYNNFKVSYENYTVKVTDSTLGTTTDKTLATDKEETYKVDFFSPADKTKAVHTAKVIVGDEKTMMVNLAEGATVIGGSADPVNARKVFDGQLGSETDNISLGWDSKQSIIFKLKEDGLIKHWRFFNDSARNPETTNKPIQEASLQIFNIKDYNLDNLLENPNKFDDEKYWITVDTYSAQGERATAFSNTLNNITSKYWRVVFDTKGDRYSSPVVPELQILGYPLPNADTIMKTVTTAKELSQQKDKFSQKMLDELKIKEMALETSLNSKIFDVTAINANAGVLKDCIEKRQLLKK

SEQ ID NO: 18 - protein, 561 aa, Artificial Sequence
  1-344 of Lactobacillus casei alfa-1,6-fucosidase with CPD tag and a  C-terminal His tag
MNDNVAWFKQAKYGMMIHWGLYSLLAGEYRGESSSAYAEWIQSKFQIPNAEYGNLATAFNPLYFDAKKIVALAKQCGMQYLVVTTKHHDGFAMYHSKVDAYNVYDATPFHRDIIGELAEACQKAGLKFGLYYSQDLDWHDPNGGGYKSNDVETAGTTWDNSWDFPDEDQKNFDLCFDNKILPQIKEIMSNYGDIATAWFDVPMTLSEAQSQTIYDTVRELQPNCLINSRLGNGKYDFVSLGDNEIPKNKEDMNKTDVDYNEITGFKPSPLGLYETAGTINDSWGFSYHDQNWKTPRTLYRYKQHLNDFGINYLLNVGLDPLGRVPMMAEENLLAAKALEDEANRALADGKILHNQNVNSWGPITVTPTTDGGETRFDGQIIVQMENDPVVAKAAANLAGKHAESSVVVQLDSDGNYRVVYGDPSKLDGKLRWQLVGHGRDHSETNNTRLSGYSADELAVKLAKFQQSFNQAENINNKPDHISIVGCSLVSDDKQKGFGHQFINAMDANGLRVDVSVRSSELAVDEAGRKHTKDANGDWVQKAENNKVSLSWDAQGHHHHHH

SEQ ID NO: 19 - protein, 214 aa, Artificial Sequence
  Light chain of Trastuzumab
DIQMTQSPSSLSASVGDRVTITCRASQDVNTAVAWYQQKPGKAPKLLIYSASFLYSGVPSRFSGSRSGTDFTLTISSLQPEDFATYYCQQHYTTPPTFGQGTKVEIKRTVAAPSVFIFPPSDEQLKSGTASVVCLLNNFYPREAKVQWKVDNALQSGNSQESVTEQDSKDSTYSLSSTLTLSKADYEKHKVYACEVTHQGLSSPVTKSFNRGEC

SEQ ID NO: 20 - protein, 450 aa, Artificial Sequence
  Heavy chain of Trastuzumab
EVQLVESGGGLVQPGGSLRLSCAASGFNIKDTYIHWVRQAPGKGLEWVARIYPTNGYTRYADSVKGRFTISADTSKNTAYLQMNSLRAEDTAVYYCSRWGGDGFYAMDYWGQGTLVTVSSASTKGPSVFPLAPSSKSTSGGTAALGCLVKDYFPEPVTVSWNSGALTSGVHTFPAVLQSSGLYSLSSVVTVPSSSLGTQTYICNVNHKPSNTKVDKKVEPKSCDKTHTCPPCPAPELLGGPSVFLFPPKPKDTLMISRTPEVTCVVVDVSHEDPEVKFNWYVDGVEVHNAKTKPREEQYNSTYRVVSVLTVLHQDWLNGKEYKCKVSNKALPAPIEKTISKAKGQPREPQVYTLPPSREEMTKNQVSLTCLVKGFYPSDIAVEWESNGQPENNYKTTPPVLDSDGSFFLYSKLTVDKSRWQQGNVFSCSVMHEALHNHYTQKSLSLSPGK

SEQ ID NO: 21 - protein, 213 aa, Artificial Sequence
  Light chain of Rituximab
QIVLSQSPAILSASPGEKVTMTCRASSSVSYIHWFQQKPGSSPKPWIYATSNLASGVPVRFSGSGSGTSYSLTISRVEAEDAATYYCQQWTSNPPTFGGGTKLEIKRTVAAPSVFIFPPSDEQLKSGTASVVCLLNNFYPREAKVQWKVDNALQSGNSQESVTEQDSKDSTYSLSSTLTLSKADYEKHKVYACEVTHQGLSSPVTKSFNRGEC

SEQ ID NO: 22 - protein, 451 aa, Artificial Sequence
  Heavy chain of Rituximab
QVQLQQPGAELVKPGASVKMSCKASGYTFTSYNMHWVKQTPGRGLEWIGAIYPGNGDTSYNQKFKGKATLTADKSSSTAYMQLSSLTSEDSAVYYCARSTYYGGDWYFNVWGAGTTVTVASASTKGPSVFPLAPSSKSTSGGTAALGCLVKDYFPEPVTVSWNSGALTSGVHTFPAVLQSSGLYSLSSVVTVPSSSLGTQTYICNVNHKPSNTKVDKKAEPKSCDKTHTCPPCPAPELLGGPSVFLFPPKPKDTLMISRTPEVTCVVVDVSHEDPEVKFNWYVDGVEVHNAKTKPREEQYNSTYRVVSVLTVLHQDWLNGKEYKCKVSNKALPAPIEKTISKAKGQPREPQVYTLPPSRDELTKNQVSLTCLVKGFYPSDIAVEWESNGQPENNYKTTPPVLDSDGSFFLYSKLTVDKSRWQQGNVFSCSVMHEALHNHYTQKSLSLSPGK

SEQ ID NO: 23 - protein, 215 aa, Artificial Sequence
  Light chain of Durvalumab
EIVLTQSPGTLSLSPGERATLSCRASQRVSSSYLAWYQQKPGQAPRLLIYDASSRATGIPDRFSGSGSGTDFTLTISRLEPEDFAVYYCQQYGSLPWTFGQGTKVEIKRTVAAPSVFIFPPSDEQLKSGTASVVCLLNNFYPREAKVQWKVDNALQSGNSQESVTEQDSKDSTYSLSSTLTLSKADYEKHKVYACEVTHQGLSSPVTKSFNRGEC

SEQ ID NO: 24 - protein, 451 aa, Artificial Sequence
  Heavy chain of Durvalumab
EVQLVESGGGLVQPGGSLRLSCAASGFTFSRYWMSWVRQAPGKGLEWVANIKQDGSEKYYVDSVKGRFTISRDNAKNSLYLQMNSLRAEDTAVYYCAREGGWFGELAFDYWGQGTLVTVSSASTKGPSVFPLAPSSKSTSGGTAALGCLVKDYFPEPVTVSWNSGALTSGVHTFPAVLQSSGLYSLSSVVTVPSSSLGTQTYICNVNHKPSNTKVDKRVEPKSCDKTHTCPPCPAPEFEGGPSVFLFPPKPKDTLMISRTPEVTCVVVDVSHEDPEVKFNWYVDGVEVHNAKTKPREEQYNSTYRVVSVLTVLHQDWLNGKEYKCKVSNKALPASIEKTISKAKGQPREPQVYTLPPSREEMTKNQVSLTCLVKGFYPSDIAVEWESNGQPENNYKTTPPVLDSDGSFFLYSKLTVDKSRWQQGNVFSCSVMHEALHNHYTQKSLSLSPGK

SEQ ID NO: 25 - DNA, 1155 bp, Artificial Sequence
  Nucleotide sequence encoding the catalytic domain and 3 heptapeptide repeats
atgttccaacccctattagacgcctttatagaaagcgcttccattgaaaaaatggtctctaaatctccccccccccccctaaaaatcgctgtggcgaattggtggggagatgaagaaattaaagaatttaaaaagagcgttctttattttatcctaagccaacgctacgcaatcaccctccaccaaaaccccaatgaatcttcagatctagtttttagcaatcctcttggagcggctagaaagattttatcttatcaaaacactaaacgagtgttttacaccggtgaaaacgaatcacctaatttcaacctctttgattacgccataggctttgatgaattggattttaatgatcgttatttgagaatgcctttgtattatgcccatttgcactatgaagccgagcttgttaatgacaccactgcgccctacaaactcaaagacaacagcctttatgctttaaaaaaaccctctcatcattttaaagaaaaccaccctaatttgtgcgcagtagtgaatgatgagagcgatcttttaaaaagagggtttgccagttttgtagcgagcaacgctaacgctcctatgaggaacgctttttatgacgctctaaattccatagagccagttactgggggaggaagtgtgagaaacactttaggctataaggttggaaacaaaagcgagtttttaagccaatacaagttcaatctctgttttgaaaactcgcaaggttatggctatgtaaccgaaaaaatccttgatgcgtattttagccataccattcctatttattgggggagtcccagcgtggcgaaagattttaaccctaaaagttttgtgaatgtgcatgatttcaacaactttgatgaagcgattgattatatcaaatacctgcacacgcacccaaacgcttatttagacatgctctatgaaaaccctttaaacacccttgatgggaaagcttacttttaccaagatttgagttttaaaaaaatcctagatttttttaaaacgattttagaaaacgacacgatttatcacaataaccctttcattttctatcgtgatctgcatgagcctttaatatctattgatgatttgagggttaattatgatgatttgagggttaattatgatgatttgagggttaattat

SEQ ID NO: 26 - DNA, 1179 bp, Artificial Sequence
  Nucleotide sequence encoding HpFT-3HR
atgttccaacccctattagacgcctttatagaaagcgcttccattgaaaaaatggtctctaaatctccccccccccccctaaaaatcgctgtggcgaattggtggggagatgaagaaattaaagaatttaaaaagagcgttctttattttatcctaagccaacgctacgcaatcaccctccaccaaaaccccaatgaatcttcagatctagtttttagcaatcctcttggagcggctagaaagattttatcttatcaaaacactaaacgagtgttttacaccggtgaaaacgaatcacctaatttcaacctctttgattacgccataggctttgatgaattggattttaatgatcgttatttgagaatgcctttgtattatgcccatttgcactatgaagccgagcttgttaatgacaccactgcgccctacaaactcaaagacaacagcctttatgctttaaaaaaaccctctcatcattttaaagaaaaccaccctaatttgtgcgcagtagtgaatgatgagagcgatcttttaaaaagagggtttgccagttttgtagcgagcaacgctaacgctcctatgaggaacgctttttatgacgctctaaattccatagagccagttactgggggaggaagtgtgagaaacactttaggctataaggttggaaacaaaagcgagtttttaagccaatacaagttcaatctctgttttgaaaactcgcaaggttatggctatgtaaccgaaaaaatccttgatgcgtattttagccataccattcctatttattgggggagtcccagcgtggcgaaagattttaaccctaaaagttttgtgaatgtgcatgatttcaacaactttgatgaagcgattgattatatcaaatacctgcacacgcacccaaacgcttatttagacatgctctatgaaaaccctttaaacacccttgatgggaaagcttacttttaccaagatttgagttttaaaaaaatcctagatttttttaaaacgattttagaaaacgacacgatttatcacaataaccctttcattttctatcgtgatctgcatgagcctttaatatctattgatgatttgagggttaattatgatgatttgagggttaattatgatgatttgagggttaattatctcgagcaccaccaccaccaccac

SEQ ID NO: 27 - DNA, 1134 bp, Artificial Sequence
  Nucleotide sequence encoding the catalytic domain and 2 heptapeptide repeats
atgttccaacccctattagacgcctttatagaaagcgcttccattgaaaaaatggtctctaaatctccccccccccccctaaaaatcgctgtggcgaattggtggggagatgaagaaattaaagaatttaaaaagagcgttctttattttatcctaagccaacgctacgcaatcaccctccaccaaaaccccaatgaatcttcagatctagtttttagcaatcctcttggagcggctagaaagattttatcttatcaaaacactaaacgagtgttttacaccggtgaaaacgaatcacctaatttcaacctctttgattacgccataggctttgatgaattggattttaatgatcgttatttgagaatgcctttgtattatgcccatttgcactatgaagccgagcttgttaatgacaccactgcgccctacaaactcaaagacaacagcctttatgctttaaaaaaaccctctcatcattttaaagaaaaccaccctaatttgtgcgcagtagtgaatgatgagagcgatcttttaaaaagagggtttgccagttttgtagcgagcaacgctaacgctcctatgaggaacgctttttatgacgctctaaattccatagagccagttactgggggaggaagtgtgagaaacactttaggctataaggttggaaacaaaagcgagtttttaagccaatacaagttcaatctctgttttgaaaactcgcaaggttatggctatgtaaccgaaaaaatccttgatgcgtattttagccataccattcctatttattgggggagtcccagcgtggcgaaagattttaaccctaaaagttttgtgaatgtgcatgatttcaacaactttgatgaagcgattgattatatcaaatacctgcacacgcacccaaacgcttatttagacatgctctatgaaaaccctttaaacacccttgatgggaaagcttacttttaccaagatttgagttttaaaaaaatcctagatttttttaaaacgattttagaaaacgacacgatttatcacaataaccctttcattttctatcgtgatctgcatgagcctttaatatctattgatgatttgagggttaattatgatgatttgagggttaattat

SEQ ID NO: 28 - DNA, 1158 bp, Artificial Sequence
  Nucleotide sequence encoding HpFT-2HR
atgttccaacccctattagacgcctttatagaaagcgcttccattgaaaaaatggtctctaaatctccccccccccccctaaaaatcgctgtggcgaattggtggggagatgaagaaattaaagaatttaaaaagagcgttctttattttatcctaagccaacgctacgcaatcaccctccaccaaaaccccaatgaatcttcagatctagtttttagcaatcctcttggagcggctagaaagattttatcttatcaaaacactaaacgagtgttttacaccggtgaaaacgaatcacctaatttcaacctctttgattacgccataggctttgatgaattggattttaatgatcgttatttgagaatgcctttgtattatgcccatttgcactatgaagccgagcttgttaatgacaccactgcgccctacaaactcaaagacaacagcctttatgctttaaaaaaaccctctcatcattttaaagaaaaccaccctaatttgtgcgcagtagtgaatgatgagagcgatcttttaaaaagagggtttgccagttttgtagcgagcaacgctaacgctcctatgaggaacgctttttatgacgctctaaattccatagagccagttactgggggaggaagtgtgagaaacactttaggctataaggttggaaacaaaagcgagtttttaagccaatacaagttcaatctctgttttgaaaactcgcaaggttatggctatgtaaccgaaaaaatccttgatgcgtattttagccataccattcctatttattgggggagtcccagcgtggcgaaagattttaaccctaaaagttttgtgaatgtgcatgatttcaacaactttgatgaagcgattgattatatcaaatacctgcacacgcacccaaacgcttatttagacatgctctatgaaaaccctttaaacacccttgatgggaaagcttacttttaccaagatttgagttttaaaaaaatcctagatttttttaaaacgattttagaaaacgacacgatttatcacaataaccctttcattttctatcgtgatctgcatgagcctttaatatctattgatgatttgagggttaattatgatgatttgagggttaattatctcgagcaccaccaccaccaccac

SEQ ID NO: 29 - DNA, 1113 bp, Artificial Sequence
  Nucleotide sequence encoding the catalytic domain and 1 heptapeptide repeat
atgttccaacccctattagacgcctttatagaaagcgcttccattgaaaaaatggtctctaaatctccccccccccccctaaaaatcgctgtggcgaattggtggggagatgaagaaattaaagaatttaaaaagagcgttctttattttatcctaagccaacgctacgcaatcaccctccaccaaaaccccaatgaatcttcagatctagtttttagcaatcctcttggagcggctagaaagattttatcttatcaaaacactaaacgagtgttttacaccggtgaaaacgaatcacctaatttcaacctctttgattacgccataggctttgatgaattggattttaatgatcgttatttgagaatgcctttgtattatgcccatttgcactatgaagccgagcttgttaatgacaccactgcgccctacaaactcaaagacaacagcctttatgctttaaaaaaaccctctcatcattttaaagaaaaccaccctaatttgtgcgcagtagtgaatgatgagagcgatcttttaaaaagagggtttgccagttttgtagcgagcaacgctaacgctcctatgaggaacgctttttatgacgctctaaattccatagagccagttactgggggaggaagtgtgagaaacactttaggctataaggttggaaacaaaagcgagtttttaagccaatacaagttcaatctctgttttgaaaactcgcaaggttatggctatgtaaccgaaaaaatccttgatgcgtattttagccataccattcctatttattgggggagtcccagcgtggcgaaagattttaaccctaaaagttttgtgaatgtgcatgatttcaacaactttgatgaagcgattgattatatcaaatacctgcacacgcacccaaacgcttatttagacatgctctatgaaaaccctttaaacacccttgatgggaaagcttacttttaccaagatttgagttttaaaaaaatcctagatttttttaaaacgattttagaaaacgacacgatttatcacaataaccctttcattttctatcgtgatctgcatgagcctttaatatctattgatgatttgagggttaattat

SEQ ID NO: 30 - DNA, 1137 bp, Artificial Sequence
  Nucleotide sequence encoding HpFT-1HR
atgttccaacccctattagacgcctttatagaaagcgcttccattgaaaaaatggtctctaaatctccccccccccccctaaaaatcgctgtggcgaattggtggggagatgaagaaattaaagaatttaaaaagagcgttctttattttatcctaagccaacgctacgcaatcaccctccaccaaaaccccaatgaatcttcagatctagtttttagcaatcctcttggagcggctagaaagattttatcttatcaaaacactaaacgagtgttttacaccggtgaaaacgaatcacctaatttcaacctctttgattacgccataggctttgatgaattggattttaatgatcgttatttgagaatgcctttgtattatgcccatttgcactatgaagccgagcttgttaatgacaccactgcgccctacaaactcaaagacaacagcctttatgctttaaaaaaaccctctcatcattttaaagaaaaccaccctaatttgtgcgcagtagtgaatgatgagagcgatcttttaaaaagagggtttgccagttttgtagcgagcaacgctaacgctcctatgaggaacgctttttatgacgctctaaattccatagagccagttactgggggaggaagtgtgagaaacactttaggctataaggttggaaacaaaagcgagtttttaagccaatacaagttcaatctctgttttgaaaactcgcaaggttatggctatgtaaccgaaaaaatccttgatgcgtattttagccataccattcctatttattgggggagtcccagcgtggcgaaagattttaaccctaaaagttttgtgaatgtgcatgatttcaacaactttgatgaagcgattgattatatcaaatacctgcacacgcacccaaacgcttatttagacatgctctatgaaaaccctttaaacacccttgatgggaaagcttacttttaccaagatttgagttttaaaaaaatcctagatttttttaaaacgattttagaaaacgacacgatttatcacaataaccctttcattttctatcgtgatctgcatgagcctttaatatctattgatgatttgagggttaattatctcgagcaccaccaccaccaccac